European Patent Specification EP 3 504 243 B1, published July 24, 2024. Title: Anti-Tim-3 Antibodies and Use Thereof. Applicant: BeiGene Zhang, Tong Xue, Liu Liu, Qi Peng, Hao Wei, Min Liu, Qi Li, Kang. The sequence listing filed with the application follows.

SEQUENCE LISTING (43 sequences)

SEQ ID NO: 1 - protein, 301 aa, Homo sapiens
MFSHLPFDCVLLLLLLLLTRSSEVEYRAEVGQNAYLPCFYTPAAPGNLVPVCWGKGACPVFECGNVVLRTDERDVNYWTSRYWLNGDFRKGDVSLTIENVTLADSGIYCCRIQIPGIMNDEKFNLKLVIKPAKVTPAPTLQRDFTAAFPRMLTTRGHGPAETQTLGSLPDINLTQISTLANELRDSRLANDLRDSGATIRIGIYIGAGICAGLALALIFGALIFKWYSHSKEKIQNLSLISLANLPPSGLANAVAEGIRSEENIYTIEENVYEVEEPNEYYCYVSSRQQPSQPLGCRFAMP

SEQ ID NO: 2 - protein, 202 aa, Homo sapiens
MFSHLPFDCVLLLLLLLLTRSSEVEYRAEVGQNAYLPCFYTPAAPGNLVPVCWGKGACPVFECGNVVLRTDERDVNYWTSRYWLNGDFRKGDVSLTIENVTLADSGIYCCRIQIPGIMNDEKFNLKLVIKPAKVTPAPTLQRDFTAAFPRMLTTRGHGPAETQTLGSLPDINLTQISTLANELRDSRLANDLRDSGATIRIG

SEQ ID NO: 3 - protein, 5 aa, Mus musculus
RYAMS

SEQ ID NO: 4 - protein, 16 aa, Mus musculus
AISSGGSLYFPDSVKG

SEQ ID NO: 5 - protein, 11 aa, Mus musculus
GREADGGYFDY

SEQ ID NO: 6 - protein, 15 aa, Mus musculus
RASESVEYYGTSLMQ

SEQ ID NO: 7 - protein, 7 aa, Mus musculus
AASNVES

SEQ ID NO: 8 - protein, 9 aa, Mus musculus
QQSMKVPLT

SEQ ID NO: 9 - protein, 119 aa, Mus musculus
EVKLVESGGGLVKPGGSLKLSCAASGFTFSRYAMSWVRQIPEKRLEWVAAISSGGSLYFPDSVKGRFTISRDNARNICYLQMNSLRSDDTAMYYCARGREADGGYFDYWGQGTTLTVSS

SEQ ID NO: 10 - DNA, 357 bp, Mus musculus
gaagtgaagctggtggagtctgggggaggcttagtgaagcctggagggtccctgaaactctcctgtgcagcctctggattcactttcagtaggtatgccatgtcttgggttcgccagattccagagaagaggctggagtgggtcgcagccattagtagtggtggtagtttatactttccagacagtgtgaagggccgattcaccatctccagagataatgccaggaacatctgctacctgcaaatgaacagtctgaggtctgacgacacggccatgtattactgtgcaagaggccgggaggccgacggaggctactttgactactggggccaaggcaccactctcacagtctcctca

SEQ ID NO: 11 - protein, 111 aa, Mus musculus
DIVLTQSPASLAVSLGQRATISCRASESVEYYGTSLMQWYQQKPGQPPKLLIYAASNVESGVPARFSGSGSGTDFSLNIHPVEEDDIAMYFCQQSMKVPLTFGAGTKLELK

SEQ ID NO: 12 - DNA, 333 bp, Mus musculus
gacattgtgctcacccaatctccagcttctttggctgtgtctctagggcagagagccaccatctcctgcagagccagtgaaagtgttgaatattatggcacaagtttaatgcagtggtaccaacagaaaccaggacaaccacccaaactcctcatctatgctgcatccaacgtagaatctggggtccctgccaggtttagtggcagtgggtctgggacagacttcagcctcaacatccatcctgtggaggaggatgatattgcaatgtatttctgtcagcaaagtatgaaggttcctctcacgttcggtgctgggaccaagctggagctgaaa

SEQ ID NO: 13 - protein, 448 aa, Artificial Sequence
  ch425 heavy chain pro
EVKLVESGGGLVKPGGSLKLSCAASGFTFSRYAMSWVRQIPEKRLEWVAAISSGGSLYFPDSVKGRFTISRDNARNICYLQMNSLRSDDTAMYYCARGREADGGYFDYWGQGTTLTVSSASTKGPSVFPLAPSSKSTSGGTAALGCLVKDYFPEPVTVSWNSGALTSGVHTFPAVLQSSGLYSLSSVVTVPSSSLGTQTYICNVNHKPSNTKVDKKVEPKSCDKTHTCPPCPAPPAAGPSVFLFPPKPKDTLMISRTPEVTCVVVDVSHEDPEVKFNWYVDGVEVHNAKTKPREEQYNSTYRVVSVLTVLHQDWLNGKEYKCKVSNKALAAPIEKTISKAKGQPREPQVYTLPPSRDELTKNQVSLTCLVKGFYPSDIAVEWESNGQPENNYKTTPPVLDSDGSFFLYSKLTVDKSRWQQGNVFSCSVMHEALHNHYTQKSLSLSPGK

SEQ ID NO: 14 - DNA, 1347 bp, Artificial Sequence
  ch425 heavy chain DNA
gaagtgaagctggtggagtctgggggaggcttagtgaagcctggagggtccctgaaactctcctgtgcagcctctggattcactttcagtaggtatgccatgtcttgggttcgccagattccagagaagaggctggagtgggtcgcagccattagtagtggtggtagtttatactttccagacagtgtgaagggccgattcaccatctccagagataatgccaggaacatctgctacctgcaaatgaacagtctgaggtctgacgacacggccatgtattactgtgcaagaggccgggaggccgacggaggctactttgactactggggccaaggcaccactctcacagtctcctcagcctccaccaagggcccatcggtcttccccctggcaccctcctccaagagtacttctgggggcacagcggccctgggctgcctggtcaaggactacttccccgaaccggtgacggtgtcgtggaactcaggcgccctgaccagcggcgtgcacaccttcccggctgtcctacagtcctcaggactctactccctcagcagcgtggtgaccgtgccctccagcagcttgggcacccagacctacatctgcaacgtgaatcacaagcccagcaacaccaaggtggacaagaaagttgagcccaaatcttgtgacaaaactcacacatgcccaccgtgcccagcacctcctgctgccggaccgtcagtcttcctcttccccccaaaacccaaggacaccctcatgatctcccggacccctgaggtcacatgcgtggtggtggacgtgagccacgaagaccctgaggtcaagttcaactggtacgtggacggcgtggaggtgcataatgccaagacaaagccgcgggaggagcagtacaacagcacgtaccgtgtggtcagcgtcctcaccgtcctgcaccaggactggctgaatggcaaggagtacaagtgcaaggtctccaacaaagccctcgccgcccccatcgagaaaaccatctccaaagccaaagggcagccccgagaaccacaggtgtacaccctgcccccatcccgggatgagctgaccaagaaccaggtcagcctgacctgcctggtcaaaggcttctatcccagcgacatcgccgtggagtgggagagcaatgggcagccggagaacaactacaagaccacgcctcccgtgctggactccgacggctccttcttcctctacagcaagctcaccgtggacaagagcaggtggcagcaggggaacgtcttctcatgctccgtgatgcatgaggctctgcacaaccactacacgcagaagagcctctccctgtctccgggtaaatga

SEQ ID NO: 15 - protein, 218 aa, Artificial Sequence
  ch425 light chain pro
DIVLTQSPASLAVSLGQRATISCRASESVEYYGTSLMQWYQQKPGQPPKLLIYAASNVESGVPARFSGSGSGTDFSLNIHPVEEDDIAMYFCQQSMKVPLTFGAGTKLELKRADAAPTVSIFPPSSEQLTSGGASVVCFLNNFYPKDINVKWKIDGSERQNGVLNSWTDQDSKDSTYSMSSTLTLTKDEYERHNSYTCEATHKTSTSPIVKSFNRNEC

SEQ ID NO: 16 - DNA, 657 bp, Artificial Sequence
  ch425 light chain DNA
gacattgtgctcacccaatctccagcttctttggctgtgtctctagggcagagagccaccatctcctgcagagccagtgaaagtgttgaatattatggcacaagtttaatgcagtggtaccaacagaaaccaggacaaccacccaaactcctcatctatgctgcatccaacgtagaatctggggtccctgccaggtttagtggcagtgggtctgggacagacttcagcctcaacatccatcctgtggaggaggatgatattgcaatgtatttctgtcagcaaagtatgaaggttcctctcacgttcggtgctgggaccaagctggagctgaaacgggctgatgctgcaccaactgtatccatcttcccaccatccagtgagcagttaacatctggaggtgcctcagtcgtgtgcttcttgaacaacttctaccccaaagacatcaatgtcaagtggaagattgatggcagtgaacgacaaaatggcgtcctgaacagttggactgatcaggacagcaaagacagcacctacagcatgagcagcaccctcacgttgaccaaggacgagtatgaacgacataacagctatacctgtgaggccactcacaagacatcaacttcacccattgtcaagagcttcaacaggaatgagtgttag

SEQ ID NO: 17 - protein, 119 aa, Artificial Sequence
  hu425-1-1 VH pro
EVQLVESGGGLVQPGGSLRLSCAASGFTFSRYAMSWVRQAPGKGLEWVAAISSGGSLYFPDSVKGRFTISRDNAKNSCYLQMNSLRAEDTAVYYCARGREADGGYFDYWGQGTLVTVSS

SEQ ID NO: 18 - DNA, 357 bp, Artificial Sequence
  hu425-1-1 VH DNA
gaagtgcagctggtcgaatcagggggggggctggtgcagcctggaggcagcctgagactgtcctgcgccgcttctggcttcacctttagcagatacgccatgtcctgggtgcggcaggctcctggcaagggactggagtgggtggccgctatcagctccggcggctccctgtacttccccgattccgtgaagggccggttcaccatcagcagggacaacgccaagaacagctgctatctgcagatgaactctctgagggccgaggatacagccgtgtactattgcgctcggggcagagaagcagatggcggctacttcgactattggggccagggcaccctggtgacagtgtctagc

SEQ ID NO: 19 - protein, 111 aa, Artificial Sequence
  hu425-1-1 VK pro
DIVLTQSPATLSVSPGERATLSCRASESVEYYGTSLMQWYQQKPGQAPRLLIYAASNVESGVPARFSGSGSGTDFTLTISSLQSEDFAVYYCQQSMKVPLTFGGGTKVEIK

SEQ ID NO: 20 - DNA, 333 bp, Artificial Sequence
  hu425-1-1 VK DNA
gacatcgtcctgactcagtcccctgccactctgtcagtgagcccaggagagcgagctaccctgtcctgcagagcatccgagtctgtcgaatactatggcacctctctgatgcagtggtaccagcagaagccagggcaggctcccaggctgctgatctatgccgcttctaacgtggagagtggcgtcccagcacgcttcagtggctcagggagcggaacagactttaccctgacaattagctccctgcagagtgaagatttcgccgtgtactattgccagcagagcatgaaggtccccctgacatttggcgggggaactaaggtggagatcaaa

SEQ ID NO: 21 - protein, 329 aa, Artificial Sequence
  IgG1mf pro
ASTKGPSVFPLAPSSKSTSGGTAALGCLVKDYFPEPVTVSWNSGALTSGVHTFPAVLQSSGLYSLSSVVTVPSSSLGTQTYICNVNHKPSNTKVDKKVEPKSCDKTHTCPPCPAPPAAGPSVFLFPPKPKDTLMISRTPEVTCVVVDVSHEDPEVKFNWYVDGVEVHNAKTKPREEQYNSTYRVVSVLTVLHQDWLNGKEYKCKVSNKALAAPIEKTISKAKGQPREPQVYTLPPSRDELTKNQVSLTCLVKGFYPSDIAVEWESNGQPENNYKTTPPVLDSDGSFFLYSKLTVDKSRWQQGNVFSCSVMHEALHNHYTQKSLSLSPGK

SEQ ID NO: 22 - protein, 448 aa, Artificial Sequence
  hu425-1-1 heavy chain pro
EVQLVESGGGLVQPGGSLRLSCAASGFTFSRYAMSWVRQAPGKGLEWVAAISSGGSLYFPDSVKGRFTISRDNAKNSCYLQMNSLRAEDTAVYYCARGREADGGYFDYWGQGTLVTVSSASTKGPSVFPLAPSSKSTSGGTAALGCLVKDYFPEPVTVSWNSGALTSGVHTFPAVLQSSGLYSLSSVVTVPSSSLGTQTYICNVNHKPSNTKVDKKVEPKSCDKTHTCPPCPAPPAAGPSVFLFPPKPKDTLMISRTPEVTCVVVDVSHEDPEVKFNWYVDGVEVHNAKTKPREEQYNSTYRVVSVLTVLHQDWLNGKEYKCKVSNKALAAPIEKTISKAKGQPREPQVYTLPPSRDELTKNQVSLTCLVKGFYPSDIAVEWESNGQPENNYKTTPPVLDSDGSFFLYSKLTVDKSRWQQGNVFSCSVMHEALHNHYTQKSLSLSPGK

SEQ ID NO: 23 - DNA, 1347 bp, Artificial Sequence
  hu425-1-1 heavy chain DNA
gaagtgcagctggtcgaatcagggggggggctggtgcagcctggaggcagcctgagactgtcctgcgccgcttctggcttcacctttagcagatacgccatgtcctgggtgcggcaggctcctggcaagggactggagtgggtggccgctatcagctccggcggctccctgtacttccccgattccgtgaagggccggttcaccatcagcagggacaacgccaagaacagctgctatctgcagatgaactctctgagggccgaggatacagccgtgtactattgcgctcggggcagagaagcagatggcggctacttcgactattggggccagggcaccctggtgacagtgtctagcgctagcaccaaaggccccagcgtgtttcctctggctccatcctctaaatccacctctggcggcacagccgctctgggctgtctggtgaaggattacttcccagagcccgtgacagtgtcttggaacagcggcgccctgacctccggcgtgcacacatttcctgctgtgctgcagagctccggcctgtacagcctgtctagcgtggtgaccgtgccatcctctagcctgggcacccagacatatatctgcaacgtgaatcacaagcccagcaatacaaaggtggataagaaggtggagccaaagtcctgtgacaagacccacacatgccccccttgtcctgctccaccagctgcaggaccaagcgtgttcctgtttccacccaagcccaaggataccctgatgatctctcggaccccagaggtgacatgcgtggtggtggatgtgagccacgaggaccccgaggtgaagttcaactggtatgtggacggcgtggaggtgcacaatgctaagaccaagcccagggaggagcagtacaactccacctatagagtggtgtctgtgctgacagtgctgcaccaggattggctgaacggcaaggagtataagtgcaaggtgtccaataaggccctggccgctcctatcgagaagaccatctctaaggccaagggccagcccagagagcctcaggtgtacacactgcctccatcccgggatgagctgaccaagaaccaggtgtctctgacatgtctggtcaagggcttctatccctctgacatcgccgtggagtgggagagcaatggccagcctgagaacaattacaagaccacaccccctgtgctggattccgacggctctttctttctgtatagcaagctgaccgtggacaagtcccggtggcagcagggcaacgtgttcagctgttccgtgatgcacgaagctctgcataatcactatactcagaaatccctgtcactgtcacctggtaaatga

SEQ ID NO: 24 - protein, 218 aa, Artificial Sequence
  hu425-1-1 light chain pro
DIVLTQSPATLSVSPGERATLSCRASESVEYYGTSLMQWYQQKPGQAPRLLIYAASNVESGVPARFSGSGSGTDFTLTISSLQSEDFAVYYCQQSMKVPLTFGGGTKVEIKRTVAAPSVFIFPPSDEQLKSGTASVVCLLNNFYPREAKVQWKVDNALQSGNSQESVTEQDSKDSTYSLSSTLTLSKADYEKHKVYACEVTHQGLSSPVTKSFNRGEC

SEQ ID NO: 25 - DNA, 657 bp, Artificial Sequence
  hu425-1-1 light chain DNA
gacatcgtcctgactcagtcccctgccactctgtcagtgagcccaggagagcgagctaccctgtcctgcagagcatccgagtctgtcgaatactatggcacctctctgatgcagtggtaccagcagaagccagggcaggctcccaggctgctgatctatgccgcttctaacgtggagagtggcgtcccagcacgcttcagtggctcagggagcggaacagactttaccctgacaattagctccctgcagagtgaagatttcgccgtgtactattgccagcagagcatgaaggtccccctgacatttggcgggggaactaaggtggagatcaaacgaacagtggcagccccttccgtcttcatttttcccccttctgacgaacagctgaaatcaggaactgctagcgtggtctgtctgctgaacaatttctaccccagagaggccaaggtgcagtggaaagtcgataacgctctgcagtccggcaattctcaggagagtgtgaccgaacaggactcaaaggatagcacatattccctgtctagtactctgaccctgagcaaagcagactacgagaagcacaaagtgtatgcctgtgaagtcacacaccaggggctgagttcaccagtcaccaagagtttcaacagaggggaatgctaa

SEQ ID NO: 26 - protein, 16 aa, Artificial Sequence
  hu425-2-2 HCDR2
AISSGGSLYYPDSVKG

SEQ ID NO: 27 - protein, 9 aa, Artificial Sequence
  hu425-2-2 LCDR3
QQSLKVPLT

SEQ ID NO: 28 - protein, 119 aa, Artificial Sequence
  hu425-2-2 VH pro
EVQLVESGGGLVQPGGSLRLSCAASGFTFSRYAMSWVRQAPGKGLEWVAAISSGGSLYYPDSVKGRFTISRDNAKNTLYLQMNSLRAEDTAVYYCARGREADGGYFDYWGQGTLVTVSS

SEQ ID NO: 29 - DNA, 357 bp, Artificial Sequence
  hu425-2-2 VH DNA
gaagtgcagctggtcgaatcagggggggggctggtgcagcctggaggcagcctgagactgtcctgcgccgcttctggcttcacctttagcagatacgccatgtcctgggtgcggcaggctcctggcaagggactggagtgggtggccgctatcagctccggcggctccctgtactatcccgattccgtgaagggccggttcaccatcagcagggacaacgccaagaacacactgtatctgcagatgaactctctgagggccgaggatacagccgtgtactattgcgctcggggcagagaagcagatggcggctacttcgactattggggccagggcaccctggtgacagtgtctagc

SEQ ID NO: 30 - protein, 111 aa, Artificial Sequence
  hu425-2-2 VK pro
EIVMTQSPATLSVSPGERATLSCRASESVEYYGTSLMQWYQQKPGQAPRLLIYAASNVESGIPARFSGSGSGTEFTLTISSLQSEDFAVYYCQQSLKVPLTFGGGTKVEIK

SEQ ID NO: 31 - DNA, 333 bp, Artificial Sequence
  hu425-2-2 VK DNA
gagatcgtcatgactcagtcccctgccactctgtcagtgagcccaggagagcgagctaccctgtcctgcagagcatccgagtctgtcgaatactatggcacctctctgatgcagtggtaccagcagaagccagggcaggctcccaggctgctgatctatgccgcttctaacgtggagagtggcatcccagcacgcttcagtggctcagggagcggaacagagtttaccctgacaattagctccctgcagagtgaagatttcgccgtgtactattgccagcagagcctgaaggtccccctgacatttggcgggggaactaaggtggagatcaaa

SEQ ID NO: 32 - protein, 448 aa, Artificial Sequence
  hu425-2-2 heavy chain pro
EVQLVESGGGLVQPGGSLRLSCAASGFTFSRYAMSWVRQAPGKGLEWVAAISSGGSLYYPDSVKGRFTISRDNAKNTLYLQMNSLRAEDTAVYYCARGREADGGYFDYWGQGTLVTVSSASTKGPSVFPLAPSSKSTSGGTAALGCLVKDYFPEPVTVSWNSGALTSGVHTFPAVLQSSGLYSLSSVVTVPSSSLGTQTYICNVNHKPSNTKVDKKVEPKSCDKTHTCPPCPAPPAAGPSVFLFPPKPKDTLMISRTPEVTCVVVDVSHEDPEVKFNWYVDGVEVHNAKTKPREEQYNSTYRVVSVLTVLHQDWLNGKEYKCKVSNKALAAPIEKTISKAKGQPREPQVYTLPPSRDELTKNQVSLTCLVKGFYPSDIAVEWESNGQPENNYKTTPPVLDSDGSFFLYSKLTVDKSRWQQGNVFSCSVMHEALHNHYTQKSLSLSPGK

SEQ ID NO: 33 - DNA, 1347 bp, Artificial Sequence
  hu425-2-2 heavy chain DNA
gaagtgcagctggtcgaatcagggggggggctggtgcagcctggaggcagcctgagactgtcctgcgccgcttctggcttcacctttagcagatacgccatgtcctgggtgcggcaggctcctggcaagggactggagtgggtggccgctatcagctccggcggctccctgtactatcccgattccgtgaagggccggttcaccatcagcagggacaacgccaagaacacactgtatctgcagatgaactctctgagggccgaggatacagccgtgtactattgcgctcggggcagagaagcagatggcggctacttcgactattggggccagggcaccctggtgacagtgtctagcgctagcaccaaaggccccagcgtgtttcctctggctccatcctctaaatccacctctggcggcacagccgctctgggctgtctggtgaaggattacttcccagagcccgtgacagtgtcttggaacagcggcgccctgacctccggcgtgcacacatttcctgctgtgctgcagagctccggcctgtacagcctgtctagcgtggtgaccgtgccatcctctagcctgggcacccagacatatatctgcaacgtgaatcacaagcccagcaatacaaaggtggataagaaggtggagccaaagtcctgtgacaagacccacacatgccccccttgtcctgctccaccagctgcaggaccaagcgtgttcctgtttccacccaagcccaaggataccctgatgatctctcggaccccagaggtgacatgcgtggtggtggatgtgagccacgaggaccccgaggtgaagttcaactggtatgtggacggcgtggaggtgcacaatgctaagaccaagcccagggaggagcagtacaactccacctatagagtggtgtctgtgctgacagtgctgcaccaggattggctgaacggcaaggagtataagtgcaaggtgtccaataaggccctggccgctcctatcgagaagaccatctctaaggccaagggccagcccagagagcctcaggtgtacacactgcctccatcccgggatgagctgaccaagaaccaggtgtctctgacatgtctggtcaagggcttctatccctctgacatcgccgtggagtgggagagcaatggccagcctgagaacaattacaagaccacaccccctgtgctggattccgacggctctttctttctgtatagcaagctgaccgtggacaagtcccggtggcagcagggcaacgtgttcagctgttccgtgatgcacgaagctctgcataatcactatactcagaaatccctgtcactgtcacctggtaaatga

SEQ ID NO: 34 - protein, 218 aa, Artificial Sequence
  hu425-2-2 light chain pro
EIVMTQSPATLSVSPGERATLSCRASESVEYYGTSLMQWYQQKPGQAPRLLIYAASNVESGIPARFSGSGSGTEFTLTISSLQSEDFAVYYCQQSLKVPLTFGGGTKVEIKRTVAAPSVFIFPPSDEQLKSGTASVVCLLNNFYPREAKVQWKVDNALQSGNSQESVTEQDSKDSTYSLSSTLTLSKADYEKHKVYACEVTHQGLSSPVTKSFNRGEC

SEQ ID NO: 35 - DNA, 657 bp, Artificial Sequence
  hu425-2-2 light chain DNA
gagatcgtcatgactcagtcccctgccactctgtcagtgagcccaggagagcgagctaccctgtcctgcagagcatccgagtctgtcgaatactatggcacctctctgatgcagtggtaccagcagaagccagggcaggctcccaggctgctgatctatgccgcttctaacgtggagagtggcatcccagcacgcttcagtggctcagggagcggaacagagtttaccctgacaattagctccctgcagagtgaagatttcgccgtgtactattgccagcagagcctgaaggtccccctgacatttggcgggggaactaaggtggagatcaaacgaacagtggcagccccttccgtcttcatttttcccccttctgacgaacagctgaaatcaggaactgctagcgtggtctgtctgctgaacaatttctaccccagagaggccaaggtgcagtggaaagtcgataacgctctgcagtccggcaattctcaggagagtgtgaccgaacaggactcaaaggatagcacatattccctgtctagtactctgaccctgagcaaagcagactacgagaagcacaaagtgtatgcctgtgaagtcacacaccaggggctgagttcaccagtcaccaagagtttcaacagaggggaatgctaa

SEQ ID NO: 36 - protein, 111 aa, Artificial Sequence
  hu425-2-3b VK pro
EIVLTQSPATLSVSPGERATLSCRASESVEYYGTSLMQWYQQKPGQAPRLLIYAASNVESGIPARFSGSGSGTEFTLTISSLQSEDFAVYYCQQSLKVPLTFGGGTKVEIK

SEQ ID NO: 37 - DNA, 333 bp, Artificial Sequence
  hu425-2-3b VK DNA
gagatcgtcctgactcagtcccctgccactctgtcagtgagcccaggagagcgagctaccctgtcctgcagagcatccgagtctgtcgaatactatggcacctctctgatgcagtggtaccagcagaagccagggcaggctcccaggctgctgatctatgccgcttctaacgtggagagtggcatcccagcacgcttcagtggctcagggagcggaacagagtttaccctgacaattagctccctgcagagtgaagatttcgccgtgtactattgccagcagagcctgaaggtccccctgacatttggcgggggaactaaggtggagatcaaa

SEQ ID NO: 38 - protein, 218 aa, Artificial Sequence
  hu425-2-3b light chain pro
EIVLTQSPATLSVSPGERATLSCRASESVEYYGTSLMQWYQQKPGQAPRLLIYAASNVESGIPARFSGSGSGTEFTLTISSLQSEDFAVYYCQQSLKVPLTFGGGTKVEIKRTVAAPSVFIFPPSDEQLKSGTASVVCLLNNFYPREAKVQWKVDNALQSGNSQESVTEQDSKDSTYSLSSTLTLSKADYEKHKVYACEVTHQGLSSPVTKSFNRGEC

SEQ ID NO: 39 - DNA, 657 bp, Artificial Sequence
  hu425-2-3b light chain DNA
gagatcgtcctgactcagtcccctgccactctgtcagtgagcccaggagagcgagctaccctgtcctgcagagcatccgagtctgtcgaatactatggcacctctctgatgcagtggtaccagcagaagccagggcaggctcccaggctgctgatctatgccgcttctaacgtggagagtggcatcccagcacgcttcagtggctcagggagcggaacagagtttaccctgacaattagctccctgcagagtgaagatttcgccgtgtactattgccagcagagcctgaaggtccccctgacatttggcgggggaactaaggtggagatcaaacgaacagtggcagccccttccgtcttcatttttcccccttctgacgaacagctgaaatcaggaactgctagcgtggtctgtctgctgaacaatttctaccccagagaggccaaggtgcagtggaaagtcgataacgctctgcagtccggcaattctcaggagagtgtgaccgaacaggactcaaaggatagcacatattccctgtctagtactctgaccctgagcaaagcagactacgagaagcacaaagtgtatgcctgtgaagtcacacaccaggggctgagttcaccagtcaccaagagtttcaacagaggggaatgctaa

SEQ ID NO: 40 - protein, 118 aa, Artificial Sequences
  artificial sequences
QVQLVQSGAEVKKPGSSVKVSCKASGYTFTSYNMHWVRQAPGQGLEWMGDIYPGNGDTSYNQKFKGRVTITADKSTSTVYMELSSLRSEDTAVYYCARVGGAFPMDYWGQGTTVTVSS

SEQ ID NO: 41 - protein, 111 aa, Artificial Sequences
  artificial sequences
AIQLTQSPSSLSASVGDRVTITCRASESVEYYGTSLMQWYQQKPGKAPKLLIYAASNVESGVPSRFSGSGSGTDFTLTISSLQPEDFATYFCQQSRKDPSTFGGGTKVEIK

SEQ ID NO: 42 - protein, 114 aa, Artificial Sequences
  artificial sequences
EVQLLESGGGLVQPGGSLRLSCAAASGFTFSSYDMSWVRQAPGKGLDWVSTISGGGTYTYYQDSVKGRFTISRDNSKNTLYLQMNSLRAEDTAVYYCASMDYWGQGTTVTVSSA

SEQ ID NO: 43 - protein, 108 aa, Artificial Sequences
  artificial sequences
DIQMTQSPSSLSASVGDRVTITCRASQSIRRYLNWYHQKPGKAPKLLIYGASTLQSGVPSRFSGSGSGTDFTLTISSLQPEDFAVYYCQQSHSAPLTFGGGTKVEIKR